European Patent Specification EP 3 417 071 B1, published April 5, 2023. Title: System and Method for Targeted Depletion of Nucleic Acids. Applicant: Roche Sequencing Solutions, Inc. F. Hoffmann-La Roche AG. The sequence listing filed with the application follows.

SEQUENCE LISTING (243 sequences)

SEQ ID NO: 1 - DNA, 38 bp, Artificial Sequence
  DNA probe sequence for depletion of target RNA
ctggttgagcacagggtactttattgatggtacatgac

SEQ ID NO: 2 - DNA, 38 bp, Artificial Sequence
  DNA probe sequence for depletion of target RNA
ggtgcggctccctaggcccctcccctcttcaaggggtc

SEQ ID NO: 3 - DNA, 38 bp, Artificial Sequence
  DNA probe sequence for depletion of target RNA
catggcaactgtgaggaggggagattcagtgtggtggg

SEQ ID NO: 4 - DNA, 38 bp, Artificial Sequence
  DNA probe sequence for depletion of target RNA
actgagtgtggcagggactccccagcagtgagggtctc

SEQ ID NO: 5 - DNA, 38 bp, Artificial Sequence
  DNA probe sequence for depletion of target RNA
tcttcctcttgtgctcttgctggggctggtggtccagg

SEQ ID NO: 6 - DNA, 38 bp, Artificial Sequence
  DNA probe sequence for depletion of target RNA
tcttactccttggaggccatgtgggccatgaggtccac

SEQ ID NO: 7 - DNA, 38 bp, Artificial Sequence
  DNA probe sequence for depletion of target RNA
ccctgttgctgtagccaaattcgttgtcataccaggaa

SEQ ID NO: 8 - DNA, 38 bp, Artificial Sequence
  DNA probe sequence for depletion of target RNA
gagcttgacaaagtggtcgttgagggcaatgccagccc

SEQ ID NO: 9 - DNA, 38 bp, Artificial Sequence
  DNA probe sequence for depletion of target RNA
gcgtcaaaggtggaggagtgggtgtcgctgttgaagtc

SEQ ID NO: 10 - DNA, 38 bp, Artificial Sequence
  DNA probe sequence for depletion of target RNA
aggagaccacctggtgctcagtgtagcccaggatgccc

SEQ ID NO: 11 - DNA, 38 bp, Artificial Sequence
  DNA probe sequence for depletion of target RNA
gagggggccctccgacgcctgcttcaccaccttcttga

SEQ ID NO: 12 - DNA, 38 bp, Artificial Sequence
  DNA probe sequence for depletion of target RNA
tcatcatatttggcaggtttttctagacggcaggtcag

SEQ ID NO: 13 - DNA, 38 bp, Artificial Sequence
  DNA probe sequence for depletion of target RNA
ccaccactgacacgttggcagtggggacacggaaggcc

SEQ ID NO: 14 - DNA, 38 bp, Artificial Sequence
  DNA probe sequence for depletion of target RNA
gccagtgagcttcccgttcagctcagggatgaccttgc

SEQ ID NO: 15 - DNA, 38 bp, Artificial Sequence
  DNA probe sequence for depletion of target RNA
acagccttggcagcgccagtagaggcagggatgatgtt

SEQ ID NO: 16 - DNA, 38 bp, Artificial Sequence
  DNA probe sequence for depletion of target RNA
ggagagccccgcggccatcacgccacagtttcccggag

SEQ ID NO: 17 - DNA, 38 bp, Artificial Sequence
  DNA probe sequence for depletion of target RNA
gccatccacagtcttctgggtggcagtgatggcatgga

SEQ ID NO: 18 - DNA, 38 bp, Artificial Sequence
  DNA probe sequence for depletion of target RNA
gtggtcatgagtccttccacgataccaaagttgtcatg

SEQ ID NO: 19 - DNA, 38 bp, Artificial Sequence
  DNA probe sequence for depletion of target RNA
tgaccttggccaggggtgctaagcagttggtggtgcag

SEQ ID NO: 20 - DNA, 38 bp, Artificial Sequence
  DNA probe sequence for depletion of target RNA
ggcattgctgatgatcttgaggctgttgtcatacttct

SEQ ID NO: 21 - DNA, 38 bp, Artificial Sequence
  DNA probe sequence for depletion of target RNA
tggttcacacccatgacgaacatgggggcatcagcaga

SEQ ID NO: 22 - DNA, 38 bp, Artificial Sequence
  DNA probe sequence for depletion of target RNA
gggcagagatgatgacccttttggctcccccctgcaaa

SEQ ID NO: 23 - DNA, 38 bp, Artificial Sequence
  DNA probe sequence for depletion of target RNA
agccccagccttctccatggtggtgaagacgccagtgg

SEQ ID NO: 24 - DNA, 38 bp, Artificial Sequence
  DNA probe sequence for depletion of target RNA
tccacgacgtactcagcgccagcatcgccccacttgat

SEQ ID NO: 25 - DNA, 38 bp, Artificial Sequence
  DNA probe sequence for depletion of target RNA
tggagggatctcgctcctggaagatggtgatgggattt

SEQ ID NO: 26 - DNA, 38 bp, Artificial Sequence
  DNA probe sequence for depletion of target RNA
attgatgacaagcttcccgttctcagccttgacggtgc

SEQ ID NO: 27 - DNA, 38 bp, Artificial Sequence
  DNA probe sequence for depletion of target RNA
tggaatttgccatgggtggaatcatattggaacatgta

SEQ ID NO: 28 - DNA, 38 bp, Artificial Sequence
  DNA probe sequence for depletion of target RNA
ccatgtagttgaggtcaatgaaggggtcattgatggca

SEQ ID NO: 29 - DNA, 38 bp, Artificial Sequence
  DNA probe sequence for depletion of target RNA
aatatccactttaccagagttaaaagcagccctggtga

SEQ ID NO: 30 - DNA, 38 bp, Artificial Sequence
  DNA probe sequence for depletion of target RNA
aggcgcccaatacgaccaaatccgttgactccgacctt

SEQ ID NO: 31 - DNA, 38 bp, Artificial Sequence
  DNA probe sequence for depletion of target RNA
ccttccccatggtgtctgagcgatgtggctcggcccgc

SEQ ID NO: 32 - DNA, 38 bp, Artificial Sequence
  DNA probe sequence for depletion of target RNA
cggcgcgaacacatccggcctgcgcccgcccctgccgc

SEQ ID NO: 33 - DNA, 38 bp, Artificial Sequence
  DNA probe sequence for depletion of target RNA
tcaggccgtccctagcctcccgggtttctctccgcccg

SEQ ID NO: 34 - DNA, 38 bp, Artificial Sequence
  DNA probe sequence for depletion of target RNA
ttcacctggcgacgcaaaagaagatgcggctgactgtc

SEQ ID NO: 35 - DNA, 38 bp, Artificial Sequence
  DNA probe sequence for depletion of target RNA
acaggaggagcagagagcgaagcgggaggctgcgggct

SEQ ID NO: 36 - DNA, 38 bp, Artificial Sequence
  DNA probe sequence for depletion of target RNA
atttatagaaaccgggggcgcggcggcaggcggtgact

SEQ ID NO: 37 - DNA, 38 bp, Artificial Sequence
  DNA probe sequence for depletion of target RNA
gaccccgcctcccgccaggctcagccagtcccagccca

SEQ ID NO: 38 - DNA, 35 bp, Artificial Sequence
  DNA probe sequence for depletion of target RNA
ggtctggagctcgtcggactcagagggcctgtctt

SEQ ID NO: 39 - DNA, 35 bp, Artificial Sequence
  DNA probe sequence for depletion of target RNA
cacaatgttcttgaagaagtggactacggggtttt

SEQ ID NO: 40 - DNA, 35 bp, Artificial Sequence
  DNA probe sequence for depletion of target RNA
cagtcctctcccctttccctgcgacgggggtggtg

SEQ ID NO: 41 - DNA, 35 bp, Artificial Sequence
  DNA probe sequence for depletion of target RNA
tcctggtctctggccttcggccccccagctaaatc

SEQ ID NO: 42 - DNA, 35 bp, Artificial Sequence
  DNA probe sequence for depletion of target RNA
cttgtgagccgatttatagtcggacgctctgcctc

SEQ ID NO: 43 - DNA, 35 bp, Artificial Sequence
  DNA probe sequence for depletion of target RNA
aaaaattttggaaagcgtgccctgggcatcgactc

SEQ ID NO: 44 - DNA, 35 bp, Artificial Sequence
  DNA probe sequence for depletion of target RNA
tctagccatgggtgatccagagcgactatctcttc

SEQ ID NO: 45 - DNA, 35 bp, Artificial Sequence
  DNA probe sequence for depletion of target RNA
taagaagctgaggacaggattccggaaccaggtgg

SEQ ID NO: 46 - DNA, 35 bp, Artificial Sequence
  DNA probe sequence for depletion of target RNA
taggtaacaggggcaagtgggattaaagttttaag

SEQ ID NO: 47 - DNA, 35 bp, Artificial Sequence
  DNA probe sequence for depletion of target RNA
gtgcacaactccgcaggcattaggggaggggtcat

SEQ ID NO: 48 - DNA, 35 bp, Artificial Sequence
  DNA probe sequence for depletion of target RNA
ttggccggaaattgccggtaggctgccgtggcctg

SEQ ID NO: 49 - DNA, 35 bp, Artificial Sequence
  DNA probe sequence for depletion of target RNA
catcacatccaggctctcggaggtggctgcactgt

SEQ ID NO: 50 - DNA, 35 bp, Artificial Sequence
  DNA probe sequence for depletion of target RNA
gggacagttttaaccgttttctgttttcatgttct

SEQ ID NO: 51 - DNA, 35 bp, Artificial Sequence
  DNA probe sequence for depletion of target RNA
ctgggggcacattgcgggggaaggaacgtgatctt

SEQ ID NO: 52 - DNA, 35 bp, Artificial Sequence
  DNA probe sequence for depletion of target RNA
tggagggacgtctgtgcacctggccccctgaagac

SEQ ID NO: 53 - DNA, 35 bp, Artificial Sequence
  DNA probe sequence for depletion of target RNA
ccgcagccacggcgaaaagaaagtccaagggtgga

SEQ ID NO: 54 - DNA, 35 bp, Artificial Sequence
  DNA probe sequence for depletion of target RNA
cagctgtgtgcctccatggcagtgaccagcaaaag

SEQ ID NO: 55 - DNA, 35 bp, Artificial Sequence
  DNA probe sequence for depletion of target RNA
ggatgtcaacagtcctctctgccgcccacgtcctc

SEQ ID NO: 56 - DNA, 35 bp, Artificial Sequence
  DNA probe sequence for depletion of target RNA
tttaggaggtgagagaaggacaggaaaaaaaaaca

SEQ ID NO: 57 - DNA, 35 bp, Artificial Sequence
  DNA probe sequence for depletion of target RNA
gccactccttgactgtctaatcctgttaggaaaaa

SEQ ID NO: 58 - DNA, 35 bp, Artificial Sequence
  DNA probe sequence for depletion of target RNA
tgcccagcccgcatgtcacataccaaaagctccca

SEQ ID NO: 59 - DNA, 35 bp, Artificial Sequence
  DNA probe sequence for depletion of target RNA
gaggtggccccctctctgtgctgccccacgttgga

SEQ ID NO: 60 - DNA, 35 bp, Artificial Sequence
  DNA probe sequence for depletion of target RNA
caggtacttggatccgtgcctctgggagggtctct

SEQ ID NO: 61 - DNA, 35 bp, Artificial Sequence
  DNA probe sequence for depletion of target RNA
acgcgaattcagctaattggggtgtgtgggcagcc

SEQ ID NO: 62 - DNA, 35 bp, Artificial Sequence
  DNA probe sequence for depletion of target RNA
gccattgcccagcccacgtttgcctccttttcctc

SEQ ID NO: 63 - DNA, 35 bp, Artificial Sequence
  DNA probe sequence for depletion of target RNA
atctccatcaccaaatctccaggaagaccctgttt

SEQ ID NO: 64 - DNA, 35 bp, Artificial Sequence
  DNA probe sequence for depletion of target RNA
ccaccatgcagggcaacggtgacgtccagaggcca

SEQ ID NO: 65 - DNA, 35 bp, Artificial Sequence
  DNA probe sequence for depletion of target RNA
ggctgtggtttggaaacgaggttgttcatagaggc

SEQ ID NO: 66 - DNA, 35 bp, Artificial Sequence
  DNA probe sequence for depletion of target RNA
ccttctgctctgagtgcgcaagtcttcctggactc

SEQ ID NO: 67 - DNA, 35 bp, Artificial Sequence
  DNA probe sequence for depletion of target RNA
tatgggcgactggcgcggctgcgaggctgtctaga

SEQ ID NO: 68 - DNA, 35 bp, Artificial Sequence
  DNA probe sequence for depletion of target RNA
cactgtgcactgccgctgccagcacgcccggtcac

SEQ ID NO: 69 - DNA, 35 bp, Artificial Sequence
  DNA probe sequence for depletion of target RNA
gaagtgaatgagccggttatcttctcagggagggt

SEQ ID NO: 70 - DNA, 35 bp, Artificial Sequence
  DNA probe sequence for depletion of target RNA
caggtgcacgcctgtgcctactcgctaccacgcgt

SEQ ID NO: 71 - DNA, 35 bp, Artificial Sequence
  DNA probe sequence for depletion of target RNA
tgggaggaagccatgcctggcatggtccatggtac

SEQ ID NO: 72 - DNA, 35 bp, Artificial Sequence
  DNA probe sequence for depletion of target RNA
ggggccgtctgctcagcccgtgtgtctcggtgagt

SEQ ID NO: 73 - DNA, 35 bp, Artificial Sequence
  DNA probe sequence for depletion of target RNA
gtgttaagaaggatatggtcagaagagctctttgt

SEQ ID NO: 74 - DNA, 35 bp, Artificial Sequence
  DNA probe sequence for depletion of target RNA
gggtcagtaggttagggagggaggcgcgaaaggag

SEQ ID NO: 75 - DNA, 35 bp, Artificial Sequence
  DNA probe sequence for depletion of target RNA
tctttggaaggcctatcaatcacaggtgcgctaaa

SEQ ID NO: 76 - DNA, 35 bp, Artificial Sequence
  DNA probe sequence for depletion of target RNA
tactcctcatctccgtcctcggggagggtgatgcc

SEQ ID NO: 77 - DNA, 35 bp, Artificial Sequence
  DNA probe sequence for depletion of target RNA
gaattagaattggattaagaagacgcgttttggca

SEQ ID NO: 78 - DNA, 35 bp, Artificial Sequence
  DNA probe sequence for depletion of target RNA
gctatatattaatagacatggtattaagcccacac

SEQ ID NO: 79 - DNA, 35 bp, Artificial Sequence
  DNA probe sequence for depletion of target RNA
gtttgtgtctggagttttgttctttgtaactctct

SEQ ID NO: 80 - DNA, 35 bp, Artificial Sequence
  DNA probe sequence for depletion of target RNA
acctcagctcagcgacgcagagtgcttctgctgaa

SEQ ID NO: 81 - DNA, 35 bp, Artificial Sequence
  DNA probe sequence for depletion of target RNA
cagcacgtgctgtgtgggtgcggccacgtatggat

SEQ ID NO: 82 - DNA, 35 bp, Artificial Sequence
  DNA probe sequence for depletion of target RNA
aaagaagcgcccgatggagtcaaggatgcccgtgt

SEQ ID NO: 83 - DNA, 35 bp, Artificial Sequence
  DNA probe sequence for depletion of target RNA
ttcaatattcaggaacagtgtacactttccgttca

SEQ ID NO: 84 - DNA, 35 bp, Artificial Sequence
  DNA probe sequence for depletion of target RNA
gggtaccttgccagagccccgcttgggcgcacccc

SEQ ID NO: 85 - DNA, 35 bp, Artificial Sequence
  DNA probe sequence for depletion of target RNA
gctgcgggcatgagagggcagagggctccggcccg

SEQ ID NO: 86 - DNA, 35 bp, Artificial Sequence
  DNA probe sequence for depletion of target RNA
tgccgggtggtgtgagtccttgtacatgttgcaca

SEQ ID NO: 87 - DNA, 35 bp, Artificial Sequence
  DNA probe sequence for depletion of target RNA
ccggccgtgtgacttctggggcagggagccgtagt

SEQ ID NO: 88 - DNA, 35 bp, Artificial Sequence
  DNA probe sequence for depletion of target RNA
aatgtctttgtggtttgtagagaatagtcaacggt

SEQ ID NO: 89 - DNA, 35 bp, Artificial Sequence
  DNA probe sequence for depletion of target RNA
taaggagaagatggttaggtctacggaggctccag

SEQ ID NO: 90 - DNA, 35 bp, Artificial Sequence
  DNA probe sequence for depletion of target RNA
gatgaaattgatggcccctaagatagaggagacac

SEQ ID NO: 91 - DNA, 35 bp, Artificial Sequence
  DNA probe sequence for depletion of target RNA
ttggtattgggttatggcagggggttttatattga

SEQ ID NO: 92 - DNA, 35 bp, Artificial Sequence
  DNA probe sequence for depletion of target RNA
aagtaggactgctgtgattaggacggatcagacga

SEQ ID NO: 93 - DNA, 35 bp, Artificial Sequence
  DNA probe sequence for depletion of target RNA
tagtagtatagtgatgccagcagctaggactggga

SEQ ID NO: 94 - DNA, 35 bp, Artificial Sequence
  DNA probe sequence for depletion of target RNA
tcctccggcggggtcgaagaaggtggtgttgaggt

SEQ ID NO: 95 - DNA, 35 bp, Artificial Sequence
  DNA probe sequence for depletion of target RNA
gtgaccgaaaaatcagaataggtgttggtatagaa

SEQ ID NO: 96 - DNA, 35 bp, Artificial Sequence
  DNA probe sequence for depletion of target RNA
ggagattattccgaagcctggtaggataagaatat

SEQ ID NO: 97 - DNA, 35 bp, Artificial Sequence
  DNA probe sequence for depletion of target RNA
gtatccaaatggttctttttttccggagtagtaag

SEQ ID NO: 98 - DNA, 35 bp, Artificial Sequence
  DNA probe sequence for depletion of target RNA
aaaccctaggaagccaattgatatcatagctcaga

SEQ ID NO: 99 - DNA, 35 bp, Artificial Sequence
  DNA probe sequence for depletion of target RNA
gcctaggactccagctcatgcgccgaataataggt

SEQ ID NO: 100 - DNA, 35 bp, Artificial Sequence
  DNA probe sequence for depletion of target RNA
gtctacgtctattcctactgtaaatatatggtgtg

SEQ ID NO: 101 - DNA, 35 bp, Artificial Sequence
  DNA probe sequence for depletion of target RNA
ggggatagcgatgattatggtagcggaggtgaaat

SEQ ID NO: 102 - DNA, 35 bp, Artificial Sequence
  DNA probe sequence for depletion of target RNA
gcttccgtggagtgtggcgagtcagctaaatactt

SEQ ID NO: 103 - DNA, 35 bp, Artificial Sequence
  DNA probe sequence for depletion of target RNA
gatgaatcctagggctcagagcactgcagcagatc

SEQ ID NO: 104 - DNA, 35 bp, Artificial Sequence
  DNA probe sequence for depletion of target RNA
gtttgctaatacaatgccagtcaggccacctacgg

SEQ ID NO: 105 - DNA, 35 bp, Artificial Sequence
  DNA probe sequence for depletion of target RNA
ggctacaacgtagtacgtgtcgtgtagtacgatgt

SEQ ID NO: 106 - DNA, 35 bp, Artificial Sequence
  DNA probe sequence for depletion of target RNA
tatgatggcaaatacagctcctattgataggacat

SEQ ID NO: 107 - DNA, 35 bp, Artificial Sequence
  DNA probe sequence for depletion of target RNA
tagggtgtagcctgagaataggggaaatcagtgaa

SEQ ID NO: 108 - DNA, 35 bp, Artificial Sequence
  DNA probe sequence for depletion of target RNA
gccgatgaatatgatagtgaaatggattttggcgt

SEQ ID NO: 109 - DNA, 35 bp, Artificial Sequence
  DNA probe sequence for depletion of target RNA
tccggataggccgagaaagtgttgtgggaagaaag

SEQ ID NO: 110 - DNA, 35 bp, Artificial Sequence
  DNA probe sequence for depletion of target RNA
gcctggctggcccagctcggctcgaataaggaggc

SEQ ID NO: 111 - DNA, 35 bp, Artificial Sequence
  DNA probe sequence for depletion of target RNA
tcatgtggtgtatgcatcggggtagtccgagtaac

SEQ ID NO: 112 - DNA, 35 bp, Artificial Sequence
  DNA probe sequence for depletion of target RNA
tactgctgttagagaaatgaatgagcctacagatg

SEQ ID NO: 113 - DNA, 35 bp, Artificial Sequence
  DNA probe sequence for depletion of target RNA
tcgcttcgaagcgaaggcttctcaaatcatgaaaa

SEQ ID NO: 114 - DNA, 35 bp, Artificial Sequence
  DNA probe sequence for depletion of target RNA
tagtcactccaggtttatggagggttcttctacta

SEQ ID NO: 115 - DNA, 35 bp, Artificial Sequence
  DNA probe sequence for depletion of target RNA
gtatacgggttcttcgaatgtgtggtagggtgggg

SEQ ID NO: 116 - DNA, 35 bp, Artificial Sequence
  DNA probe sequence for depletion of target RNA
ggctgtgacgataacgttgtagatgtggtcgttac

SEQ ID NO: 117 - DNA, 35 bp, Artificial Sequence
  DNA probe sequence for depletion of target RNA
gattatgatgggtattactatgaagaagattatta

SEQ ID NO: 118 - DNA, 35 bp, Artificial Sequence
  DNA probe sequence for depletion of target RNA
gggggcaccgattattaggggaactagtcagttgc

SEQ ID NO: 119 - DNA, 35 bp, Artificial Sequence
  DNA probe sequence for depletion of target RNA
taagagtcagaagcttatgttgtttatgcggggaa

SEQ ID NO: 120 - DNA, 35 bp, Artificial Sequence
  DNA probe sequence for depletion of target RNA
ggcctccactatagcagatgcgagcaggagtagga

SEQ ID NO: 121 - DNA, 35 bp, Artificial Sequence
  DNA probe sequence for depletion of target RNA
gttccctgctaagggagggtagactgttcaacctg

SEQ ID NO: 122 - DNA, 35 bp, Artificial Sequence
  DNA probe sequence for depletion of target RNA
aggggaagtagcgtcttgtagacctacttgcgctg

SEQ ID NO: 123 - DNA, 35 bp, Artificial Sequence
  DNA probe sequence for depletion of target RNA
aatgggggcttcaatcgggagtactactcgattgt

SEQ ID NO: 124 - DNA, 35 bp, Artificial Sequence
  DNA probe sequence for depletion of target RNA
gacagctcatgagtgcaagacgtcttgtgatgtaa

SEQ ID NO: 125 - DNA, 35 bp, Artificial Sequence
  DNA probe sequence for depletion of target RNA
gtttagacgtccgggaattgcatctgtttttaagc

SEQ ID NO: 126 - DNA, 35 bp, Artificial Sequence
  DNA probe sequence for depletion of target RNA
ttgaccgtagtatacccccggtcgtgtagcggtga

SEQ ID NO: 127 - DNA, 35 bp, Artificial Sequence
  DNA probe sequence for depletion of target RNA
gacgatgggcatgaaactgtggtttgctccacaga

SEQ ID NO: 128 - DNA, 35 bp, Artificial Sequence
  DNA probe sequence for depletion of target RNA
aaatacgggccctatttcaaagatttttaggggaa

SEQ ID NO: 129 - DNA, 35 bp, Artificial Sequence
  DNA probe sequence for depletion of target RNA
gattatgagggcgtgatcatgaaaggtgataagct

SEQ ID NO: 130 - DNA, 35 bp, Artificial Sequence
  DNA probe sequence for depletion of target RNA
tgttaggaaaagggcatacaggactaggaagcaga

SEQ ID NO: 131 - DNA, 35 bp, Artificial Sequence
  DNA probe sequence for depletion of target RNA
ttcctgagcgtctgagatgttagtattagttagtt

SEQ ID NO: 132 - DNA, 35 bp, Artificial Sequence
  DNA probe sequence for depletion of target RNA
gaggactaggatgatggcgggcaggatagttcaga

SEQ ID NO: 133 - DNA, 35 bp, Artificial Sequence
  DNA probe sequence for depletion of target RNA
gacctcgtctgttatgtaaaggatgcgtagggatg

SEQ ID NO: 134 - DNA, 35 bp, Artificial Sequence
  DNA probe sequence for depletion of target RNA
gtaccattggtggccaattgatttgatggtaaggg

SEQ ID NO: 135 - DNA, 35 bp, Artificial Sequence
  DNA probe sequence for depletion of target RNA
ggagttgaagattagtccgccgtagtcggtgtact

SEQ ID NO: 136 - DNA, 35 bp, Artificial Sequence
  DNA probe sequence for depletion of target RNA
gagtcgcaggtcgcctggttctaggaataatgggg

SEQ ID NO: 137 - DNA, 35 bp, Artificial Sequence
  DNA probe sequence for depletion of target RNA
tgggctgggttttactatatgataggcatgtgatt

SEQ ID NO: 138 - DNA, 35 bp, Artificial Sequence
  DNA probe sequence for depletion of target RNA
actatggtgagctcaggtgattgatactcctgatg

SEQ ID NO: 139 - DNA, 35 bp, Artificial Sequence
  DNA probe sequence for depletion of target RNA
aataagcagtgcttgaattatttggtttcggttgt

SEQ ID NO: 140 - DNA, 35 bp, Artificial Sequence
  DNA probe sequence for depletion of target RNA
ctctgaggcttgtaggagggtaaaatagagaccca

SEQ ID NO: 141 - DNA, 35 bp, Artificial Sequence
  DNA probe sequence for depletion of target RNA
tgagccgtagatgccgtcggaaatggtgaagggag

SEQ ID NO: 142 - DNA, 35 bp, Artificial Sequence
  DNA probe sequence for depletion of target RNA
aataatgacgtgaagtccgtggaagcctgtggcta

SEQ ID NO: 143 - DNA, 35 bp, Artificial Sequence
  DNA probe sequence for depletion of target RNA
aaatattagttggcggatgaagcagatagtgagga

SEQ ID NO: 144 - DNA, 35 bp, Artificial Sequence
  DNA probe sequence for depletion of target RNA
tcaggcggcggcttcgaagccaaagtgatgtttgg

SEQ ID NO: 145 - DNA, 35 bp, Artificial Sequence
  DNA probe sequence for depletion of target RNA
ggagacatacagaaatagtcaaaccacatctacaa

SEQ ID NO: 146 - DNA, 35 bp, Artificial Sequence
  DNA probe sequence for depletion of target RNA
gccggaggtcattaggagggctgagagggcccctg

SEQ ID NO: 147 - DNA, 35 bp, Artificial Sequence
  DNA probe sequence for depletion of target RNA
tagtatgaggagcgttatggagtggaagtgaaatc

SEQ ID NO: 148 - DNA, 35 bp, Artificial Sequence
  DNA probe sequence for depletion of target RNA
atcgcgccatcattggtatatggttagtgtgttgg

SEQ ID NO: 149 - DNA, 35 bp, Artificial Sequence
  DNA probe sequence for depletion of target RNA
gacaggtggtgtgtggtggccttggtatgtgcttt

SEQ ID NO: 150 - DNA, 35 bp, Artificial Sequence
  DNA probe sequence for depletion of target RNA
ttctgaggtaataaataggattatcccgtatcgaa

SEQ ID NO: 151 - DNA, 35 bp, Artificial Sequence
  DNA probe sequence for depletion of target RNA
gctggagtggtaaaaggctcagaaaaatcctgcga

SEQ ID NO: 152 - DNA, 35 bp, Artificial Sequence
  DNA probe sequence for depletion of target RNA
gcctgttgggggccagtgccctcctaattgggggg

SEQ ID NO: 153 - DNA, 35 bp, Artificial Sequence
  DNA probe sequence for depletion of target RNA
ggatgtgtttaggagtgggacttctaggggattta

SEQ ID NO: 154 - DNA, 35 bp, Artificial Sequence
  DNA probe sequence for depletion of target RNA
ctcagtgtgtagcctaggatacaggccttcagcac

SEQ ID NO: 155 - DNA, 35 bp, Artificial Sequence
  DNA probe sequence for depletion of target RNA
cggggactttcccctaggcggaaaggggaggaaca

SEQ ID NO: 156 - DNA, 35 bp, Artificial Sequence
  DNA probe sequence for depletion of target RNA
gtctacgtgcgtatgcacgtggcactctctgcccg

SEQ ID NO: 157 - DNA, 35 bp, Artificial Sequence
  DNA probe sequence for depletion of target RNA
atacgcttcttggcggactttggagtgggaagcgg

SEQ ID NO: 158 - DNA, 35 bp, Artificial Sequence
  DNA probe sequence for depletion of target RNA
agctgacggatgacgcccccgcgccacgccgctca

SEQ ID NO: 159 - DNA, 35 bp, Artificial Sequence
  DNA probe sequence for depletion of target RNA
ggttggtgcgcggacacgcactgcctgcgtaacta

SEQ ID NO: 160 - DNA, 35 bp, Artificial Sequence
  DNA probe sequence for depletion of target RNA
atcctccagcctcagcctcccgagtagctgggact

SEQ ID NO: 161 - DNA, 35 bp, Artificial Sequence
  DNA probe sequence for depletion of target RNA
atcctcccacctcagcctcccgagtagctgggact

SEQ ID NO: 162 - DNA, 35 bp, Artificial Sequence
  DNA probe sequence for depletion of target RNA
ggcatagcgcactacagcccagaactcctggactc

SEQ ID NO: 163 - DNA, 35 bp, Artificial Sequence
  DNA probe sequence for depletion of target RNA
gtcaccatattgatgccgaacttagtgcggacacc

SEQ ID NO: 164 - DNA, 35 bp, Artificial Sequence
  DNA probe sequence for depletion of target RNA
cccctccttaggcaacctggtggtcccccgctccc

SEQ ID NO: 165 - DNA, 35 bp, Artificial Sequence
  DNA probe sequence for depletion of target RNA
ggagttttgacctgctccgtttccgacctgggccg

SEQ ID NO: 166 - DNA, 35 bp, Artificial Sequence
  DNA probe sequence for depletion of target RNA
ggagttttgacctgctctgtttccgacctgggccg

SEQ ID NO: 167 - DNA, 35 bp, Artificial Sequence
  DNA probe sequence for depletion of target RNA
gtggctattcacaggcgcgatcccactactgatca

SEQ ID NO: 168 - DNA, 35 bp, Artificial Sequence
  DNA probe sequence for depletion of target RNA
agagacggggtctcgctatgttgcccaggctggag

SEQ ID NO: 169 - DNA, 35 bp, Artificial Sequence
  DNA probe sequence for depletion of target RNA
atggggtgacagatgtcgcagccagatcgccctca

SEQ ID NO: 170 - DNA, 35 bp, Artificial Sequence
  DNA probe sequence for depletion of target RNA
gcctagccagccagatcagccgaatcaaccctggc

SEQ ID NO: 171 - DNA, 35 bp, Artificial Sequence
  DNA probe sequence for depletion of target RNA
ggggatggtcgtcctcttcgaccgagcgcgcagct

SEQ ID NO: 172 - DNA, 35 bp, Artificial Sequence
  DNA probe sequence for depletion of target RNA
tactcgtatacccttgaccgaagaccggtcctcct

SEQ ID NO: 173 - DNA, 35 bp, Artificial Sequence
  DNA probe sequence for depletion of target RNA
cttgagagcttgtttggaggttctagcaggggagc

SEQ ID NO: 174 - DNA, 35 bp, Artificial Sequence
  DNA probe sequence for depletion of target RNA
cttggaagcttgactaccctacgttctcctacaaa

SEQ ID NO: 175 - DNA, 35 bp, Artificial Sequence
  DNA probe sequence for depletion of target RNA
gactgccacatgcagcgcctcatttggatgtgtct

SEQ ID NO: 176 - DNA, 35 bp, Artificial Sequence
  DNA probe sequence for depletion of target RNA
gatactacacttgatcttagccaaaaggccgagaa

SEQ ID NO: 177 - DNA, 35 bp, Artificial Sequence
  DNA probe sequence for depletion of target RNA
gtcctcggatagaggacgtatcagatattaaactg

SEQ ID NO: 178 - DNA, 35 bp, Artificial Sequence
  DNA probe sequence for depletion of target RNA
cggagcaagctcctattccatctcctatttccaaa

SEQ ID NO: 179 - DNA, 35 bp, Artificial Sequence
  DNA probe sequence for depletion of target RNA
gtgcaccgttcctggaagtactgcaataccaggtc

SEQ ID NO: 180 - DNA, 35 bp, Artificial Sequence
  DNA probe sequence for depletion of target RNA
gcactcagctcgtggccccactgatgagcttccct

SEQ ID NO: 181 - DNA, 35 bp, Artificial Sequence
  DNA probe sequence for depletion of target RNA
tcagaccttcccaagggacatgggagtggagtgac

SEQ ID NO: 182 - DNA, 35 bp, Artificial Sequence
  DNA probe sequence for depletion of target RNA
ctcagggagagccctgttagggccgcctctggccc

SEQ ID NO: 183 - DNA, 35 bp, Artificial Sequence
  DNA probe sequence for depletion of target RNA
cgcgcggagccccgttctctgggaactcacctccc

SEQ ID NO: 184 - DNA, 35 bp, Artificial Sequence
  DNA probe sequence for depletion of target RNA
gaagggcggggtccacggcatctcctgcccagtct

SEQ ID NO: 185 - DNA, 35 bp, Artificial Sequence
  DNA probe sequence for depletion of target RNA
ctggccgtgagtctgttccaagctccggcaaagga

SEQ ID NO: 186 - DNA, 35 bp, Artificial Sequence
  DNA probe sequence for depletion of target RNA
tgcggggtacctcacctcagccattgaactcactt

SEQ ID NO: 187 - DNA, 35 bp, Artificial Sequence
  DNA probe sequence for depletion of target RNA
gcggaggagagtagtctgaattgggttatgaggtc

SEQ ID NO: 188 - DNA, 35 bp, Artificial Sequence
  DNA probe sequence for depletion of target RNA
cgcctgacctccccgaggtttcgtcttcaatgcaa

SEQ ID NO: 189 - DNA, 35 bp, Artificial Sequence
  DNA probe sequence for depletion of target RNA
ctgatggccatctgctcccgttcgtccactacacg

SEQ ID NO: 190 - DNA, 35 bp, Artificial Sequence
  DNA probe sequence for depletion of target RNA
tcattgcccatatccagggccatgtgacggaggtt

SEQ ID NO: 191 - DNA, 35 bp, Artificial Sequence
  DNA probe sequence for depletion of target RNA
gttttgttggaatcagccttctccatgatcctgtc

SEQ ID NO: 192 - DNA, 35 bp, Artificial Sequence
  DNA probe sequence for depletion of target RNA
gggcacacttaaccacttcccagcatctttgttgc

SEQ ID NO: 193 - DNA, 35 bp, Artificial Sequence
  DNA probe sequence for depletion of target RNA
gacaacattcacaatgggggtggactgatgtgtgt

SEQ ID NO: 194 - DNA, 35 bp, Artificial Sequence
  DNA probe sequence for depletion of target RNA
aagagaccaagagagaacaaaagacacaaagtatt

SEQ ID NO: 195 - DNA, 35 bp, Artificial Sequence
  DNA probe sequence for depletion of target RNA
actcaagacctcaaggagttagagccaccaaatga

SEQ ID NO: 196 - DNA, 35 bp, Artificial Sequence
  DNA probe sequence for depletion of target RNA
cgggcctctgcaggttgcaactgtggtggagccgc

SEQ ID NO: 197 - DNA, 35 bp, Artificial Sequence
  DNA probe sequence for depletion of target RNA
gtggaatgtcacagttttacaagaacaatactgtg

SEQ ID NO: 198 - DNA, 35 bp, Artificial Sequence
  DNA probe sequence for depletion of target RNA
aagacggcacattttgagagattcagagcctgaca

SEQ ID NO: 199 - DNA, 35 bp, Artificial Sequence
  DNA probe sequence for depletion of target RNA
tgtaattccacattgtctaatcatgaaatcataaa

SEQ ID NO: 200 - DNA, 35 bp, Artificial Sequence
  DNA probe sequence for depletion of target RNA
tgttgtctcatcagtatgctactgtcatggaaagt

SEQ ID NO: 201 - DNA, 35 bp, Artificial Sequence
  DNA probe sequence for depletion of target RNA
caatactgagcatgctttgttgttgttctgttgtt

SEQ ID NO: 202 - DNA, 35 bp, Artificial Sequence
  DNA probe sequence for depletion of target RNA
gacaggaaaaaagtgacactactgcacttttgctg

SEQ ID NO: 203 - DNA, 35 bp, Artificial Sequence
  DNA probe sequence for depletion of target RNA
aatttcagccaaacatatattttgctggaaatgat

SEQ ID NO: 204 - DNA, 35 bp, Artificial Sequence
  DNA probe sequence for depletion of target RNA
ctctccaaaacatagccatcaaaagcagcaaacaa

SEQ ID NO: 205 - DNA, 35 bp, Artificial Sequence
  DNA probe sequence for depletion of target RNA
tggttagtaagagtcagccttataaaatttacatc

SEQ ID NO: 206 - DNA, 35 bp, Artificial Sequence
  DNA probe sequence for depletion of target RNA
aggaggaatttaatattacatgctataatgatatt

SEQ ID NO: 207 - DNA, 35 bp, Artificial Sequence
  DNA probe sequence for depletion of target RNA
ttttaataattttaaactagctacaaaatgtcaat

SEQ ID NO: 208 - DNA, 35 bp, Artificial Sequence
  DNA probe sequence for depletion of target RNA
tcattgcgcatgtctgcgtcttcggccatggtagc

SEQ ID NO: 209 - DNA, 35 bp, Artificial Sequence
  DNA probe sequence for depletion of target RNA
cgggtgctttccagcgactcatcagccaactggtc

SEQ ID NO: 210 - DNA, 35 bp, Artificial Sequence
  DNA probe sequence for depletion of target RNA
aacataaccaaagtcctgataccagcatctttact

SEQ ID NO: 211 - DNA, 35 bp, Artificial Sequence
  DNA probe sequence for depletion of target RNA
cacacacaaagcccgcagaattttcctaggtccgt

SEQ ID NO: 212 - DNA, 35 bp, Artificial Sequence
  DNA probe sequence for depletion of target RNA
tcctgattattgccccaggcttttttgtaagcatc

SEQ ID NO: 213 - DNA, 35 bp, Artificial Sequence
  DNA probe sequence for depletion of target RNA
agtaacacactatagaaatgatccctgaaagtata

SEQ ID NO: 214 - DNA, 35 bp, Artificial Sequence
  DNA probe sequence for depletion of target RNA
cagcatcccccgcctcgcgccaagactaaaattaa

SEQ ID NO: 215 - DNA, 35 bp, Artificial Sequence
  DNA probe sequence for depletion of target RNA
atgggagaaaacgcaaaaagagacaataggaggtg

SEQ ID NO: 216 - DNA, 35 bp, Artificial Sequence
  DNA probe sequence for depletion of target RNA
gagtggcgggcgggaaacggcgacaaaagagggag

SEQ ID NO: 217 - DNA, 35 bp, Artificial Sequence
  DNA probe sequence for depletion of target RNA
cagacagaacaagagacccggagaccccgtctggg

SEQ ID NO: 218 - DNA, 35 bp, Artificial Sequence
  DNA probe sequence for depletion of target RNA
aggagccgagatcgcgccactgcaatccagccggg

SEQ ID NO: 219 - DNA, 35 bp, Artificial Sequence
  DNA probe sequence for depletion of target RNA
aggcgggagactcgcttgagcccgggaggcagatg

SEQ ID NO: 220 - DNA, 35 bp, Artificial Sequence
  DNA probe sequence for depletion of target RNA
ggcgtgtgcgcctttaagccccggctactcgggag

SEQ ID NO: 221 - DNA, 35 bp, Artificial Sequence
  DNA probe sequence for depletion of target RNA
cgtggttttcggtgctctacacgttcagagaaact

SEQ ID NO: 222 - DNA, 35 bp, Artificial Sequence
  DNA probe sequence for depletion of target RNA
gccggcttcacgctcaggagaaaacgctacctctc

SEQ ID NO: 223 - DNA, 35 bp, Artificial Sequence
  DNA probe sequence for depletion of target RNA
tcaatggctgacggcagttgcagccaagcaacgcc

SEQ ID NO: 224 - DNA, 35 bp, Artificial Sequence
  DNA probe sequence for depletion of target RNA
ctctccctctcactccccaatacggagagaagaac

SEQ ID NO: 225 - DNA, 35 bp, Artificial Sequence
  DNA probe sequence for depletion of target RNA
cattgagccatcaagaaggaaaaaccactcagacc

SEQ ID NO: 226 - DNA, 35 bp, Artificial Sequence
  DNA probe sequence for depletion of target RNA
cagcccagaaacgccccggagtttacgagctagtc

SEQ ID NO: 227 - DNA, 35 bp, Artificial Sequence
  DNA probe sequence for depletion of target RNA
aggcgaaaacctttctcgcgacatgccaagcagga

SEQ ID NO: 228 - DNA, 35 bp, Artificial Sequence
  DNA probe sequence for depletion of target RNA
caccccgagaaaacccaagagccgtcaccgctgaa

SEQ ID NO: 229 - DNA, 299 bp, Homo sapiens
gccgggcgcggtggcgcgtgcctgtagtcccagctactcgggaggctgaggctggaggatcgcttgagtccaggagttctgggctgtagtgcgctatgccgatcgggtgtccgcactaagttcggcatcaatatggtgacctcccgggagcgggggaccaccaggttgcctaaggaggggtgaaccggcccaggtcggaaacggagcaggtcaaaactcccgtgctgatcagtagtgggatcgcgcctgtgaatagccactgcactccagcctgggcaacatagcgagaccccgtctct

SEQ ID NO: 230 - DNA, 332 bp, Homo sapiens
ggatgtgagggcgatctggctgcgacatctgtcaccccattgatcgccagggttgattcggctgatctggctggctaggcgggtgtccccttcctccctcaccgctccatgtgcgtccctcccgaagctgcgcgctcggtcgaagaggacgaccatccccgatagaggaggaccggtcttcggtcaagggtatacgagtagctgcgctcccctgctagaacctccaaacaagctctcaaggtccatttgtaggagaacgtagggtagtcaagcttccaagactccagacacatccaaatgaggcgctgcatgtggcagtctgcctttctttt

SEQ ID NO: 231 - DNA, 295 bp, Homo sapiens
gccgggcacagtggcgcgtgcctgtagtcccagctactcgggaggctgaggtgggaggatcgcttgagcccaggagttctgggctgtagtgcgctatgccgatcgggtgtccgcactaagttcggcatcaatatggtgacctcccgggagcgggggaccaccaggttgcctaaggaggggtgaaccggcccaggtcggaaacagagcaggtcaaaactcccgtgctgatcaggagacagagtttgtgagcagacaactggtctgaccaaaatttatgaggtgggaatttcctctt

SEQ ID NO: 232 - DNA, 321 bp, Homo sapiens
gccgggcgcggtggcgcgtgcctgtggtcccagctactcgggaggctgaggctggaggatcgcttgagtccaggagttctgggctgtagtgcgctatgccgatcgggtgtccgcactaagttcggcatcaatatggtgacctcccgggagcgggggaccaccaggttgcctaaggaggggtgaaccggcccaggtcggaaacggagcaggtcaaaactcccgtgctgatcagtagaagtctgtaatgctactggtgtcccctaattttcttatagccacagttcctttcgcctgagctcattacagagacaaatatccatt

SEQ ID NO: 233 - DNA, 333 bp, Homo sapiens
ggcggagggaagctcatcagtggggccacgagctgagtgcgtcctgtcactccactcccatgtcccttgggaaggtctgagactagggccagaggcggccctaacagggctctccctgagcttcggggaggtgagttcccagagaacggggctccgcgcgaggtcagactgggcaggagatgccgtggaccccgcccttcggggaggggcccggcggatgcctcctttgccggagcttggaacagactcacggccagcgaagtgagttcaatggctgaggtgaggtaccccgcaggggacctcataacccaattcagactactctcctccgcc

SEQ ID NO: 234 - DNA, 277 bp, Homo sapiens
ggttcgtgctgaaggcctgtatcctaggctacacactgaggactctgttcctcccctttccgcctaggggaaagtccccggacctcgggcagagagtgccacgtgcatacgcacgtagacattccccgcttcccactccaaagtccgccaagaagcgtatcccgctgagcggcgtggcgcgggggcgtcatccgtcagctccctctagttacgcaggcagtgcgtgtccgcgcaccaaccacacggggctcattctcagcgcggctgtaaaaaaaaa

SEQ ID NO: 235 - DNA, 191 bp, Homo sapiens
atcgcttctcggccttttggctaagatcaagtgtagtatctgttcttatcagtttaatatctgatacgtcctctatccgaggacaatatattaaatggatttttggaaataggagatggaataggagcttgctccgtccactccacgcatcgacctggtattgcagtacttccaggaacggtgcactctcc

SEQ ID NO: 236 - DNA, 699 bp, Homo sapiens
aagactatactttcagggatcatttctatagtgtgttactagagaagtttctctgaacgtgtagagcaccgaaaaccacgaggaagagaggtagcgttttctcctgagcgtgaagccggctttctggcgttgcttggctgcaactgccgtcagccattgatgatcgttcttctctccgtattggggagtgagagggagagaacgcggtctgagtggtttttccttcttgatggctcaatgacagagactagctcgtaaactccggggcgtttctgggctgttcgctcctgcttggcatgtcgcgagaaaggttttcgcctcctgtttcagcggtgacggctcttgggttttctcggggtggctttttaattttagtcttggcgcgaggcgggggatgctgtgtggcacctcctattgtctctttttgcgttttctcccattctcgctccctcttttgtcgccgtttcccgcccgccactcccacccccagacggggtctccgggtctcttgttctgtctgccggccccggctggattgcagtggcgcgatctcggctcctagcaacatctgcctcccgggctcaagcgagtctcccgcctaagccctcccgagtagccggggcttaaaggcgcacacgccactccaggctttttttttttttttttttttttttttggcagaaacggggtgtcagcatg

SEQ ID NO: 237 - DNA, 1542 bp, Homo sapiens
atgttcgccgaccgttgactattctctacaaaccacaaagacattggaacactatacctattattcggcgcatgagctggagtcctaggcacagctctaagcctccttattcgagccgagctgggccagccaggcaaccttctaggtaacgaccacatctacaacgttatcgtcacagcccatgcatttgtaataatcttcttcatagtaatacccatcataatcggaggctttggcaactgactagttcccctaataatcggtgcccccgatatggcgtttccccgcataaacaacataagcttctgactcttacctccctctctcctactcctgctcgcatctgctatagtggaggccggagcaggaacaggttgaacagtctaccctcccttagcagggaactactcccaccctggagcctccgtagacctaaccatcttctccttacacctagcaggtgtctcctctatcttaggggccatcaatttcatcacaacaattatcaatataaaaccccctgccataacccaataccaaacgcccctcttcgtctgatccgtcctaatcacagcagtcctacttctcctatctctcccagtcctagctgctggcatcactatactactaacagaccgcaacctcaacaccaccttcttcgaccccgccggaggaggagaccccattctataccaacacctattctgatttttcggtcaccctgaagtttatattcttatcctaccaggcttcggaataatctcccatattgtaacttactactccggaaaaaaagaaccatttggatacataggtatggtctgagctatgatatcaattggcttcctagggtttatcgtgtgagcacaccatatatttacagtaggaatagacgtagacacacgagcatatttcacctccgctaccataatcatcgctatccccaccggcgtcaaagtatttagctgactcgccacactccacggaagcaatatgaaatgatctgctgcagtgctctgagccctaggattcatctttcttttcaccgtaggtggcctgactggcattgtattagcaaactcatcactagacatcgtactacacgacacgtactacgttgtagcccacttccactatgtcctatcaataggagctgtatttgccatcataggaggcttcattcactgatttcccctattctcaggctacaccctagaccaaacctacgccaaaatccatttcactatcatattcatcggcgtaaatctaactttcttcccacaacactttctcggcctatccggaatgccccgacgttactcggactaccccgatgcatacaccacatgaaacatcctatcatctgtaggctcattcatttctctaacagcagtaatattaataattttcatgatttgagaagccttcgcttcgaagcgaaaagtcctaatagtagaagaaccctccataaacctggagtgactatatggatgccccccaccctaccacacattcgaagaacccgtatacataaaatctaga

SEQ ID NO: 238 - DNA, 784 bp, Homo sapiens
atgacccaccaatcacatgcctatcatatagtaaaacccagcccatgacccctaacaggggccctctcagccctcctaatgacctccggcctagccatgtgatttcacttccactccataacgctcctcatactaggcctactaaccaacacactaaccatataccaatgatggcgcgatgtaacacgagaaagcacataccaaggccaccacacaccacctgtccaaaaaggccttcgatacgggataatcctatttattacctcagaagtttttttcttcgcaggatttttctgagccttttaccactccagcctagcccctaccccccaattaggagggcactggcccccaacaggcatcaccccgctaaatcccctagaagtcccactcctaaacacatccgtattactcgcatcaggagtatcaatcacctgagctcaccatagtctaatagaaaacaaccgaaaccaaataattcaagcactgcttattacaattttactgggtctctattttaccctcctacaagcctcagagtacttcgagtctcccttcaccatttccgacggcatctacggctcaacattttttgtagccacaggcttccacggacttcacgtcattattggctcaactttcctcactatctgcttcatccgccaactaatatttcactttacatccaaacatcactttggcttcgaagccgccgcctgatactggcattttgtagatgtggtttgactatttctgtatgtctccatctattgatgagggtctt

SEQ ID NO: 239 - DNA, 684 bp, Homo sapiens
atggcacatgcagcgcaagtaggtctacaagacgctacttcccctatcatagaagagcttatcacctttcatgatcacgccctcataatcattttccttatctgcttcctagtcctgtatgcccttttcctaacactcacaacaaaactaactaatactaacatctcagacgctcaggaaatagaaaccgtctgaactatcctgcccgccatcatcctagtcctcatcgccctcccatccctacgcatcctttacataacagacgaggtcaacgatccctcccttaccatcaaatcaattggccaccaatggtactgaacctacgagtacaccgactacggcggactaatcttcaactcctacatacttcccccattattcctagaaccaggcgacctgcgactccttgacgttgacaatcgagtagtactcccgattgaagcccccattcgtataataattacatcacaagacgtcttgcactcatgagctgtccccacattaggcttaaaaacagatgcaattcccggacgtctaaaccaaaccactttcaccgctacacgaccgggggtatactacggtcaatgctctgaaatctgtggagcaaaccacagtttcatgcccatcgtcctagaattaattcccctaaaaatctttgaaatagggcccgtatttaccctatag

SEQ ID NO: 240 - DNA, 2300 bp, Homo sapiens
ggacaacaccttcaaagacaggccctctgagtccgacgagctccagaccatccaagaagacagtgcagccacctccgagagcctggatgtgatggcgtcacagaagagaccctcccagaggcacggatccaagtacctggccacagcaagtaccatggaccatgccaggcatggcttcctcccaaggcacagagacacgggcatccttgactccatcgggcgcttctttggcggtgacaggggtgcgcccaagcggggctctggcaaggtaccctggctaaagccgggccggagccctctgccctctcatgcccgcagccagcctgggctgtgcaacatgtacaaggactcacaccacccggcaagaactgctcactacggctccctgccccagaagtcacacggccggacccaagatgaaaaccccgtagtccacttcttcaagaacattgtgacgcctcgcacaccacccccgtcgcagggaaaggggagaggactgtccctgagcagatttagctggggggccgaaggccagagaccaggatttggctacggaggcagagcgtccgactataaatcggctcacaagggattcaagggagtcgatgcccagggcacgctttccaaaatttttaagctgggaggaagagatagtcgctctggatcacccatggctagacgctgaaaacccacctggttccggaatcctgtcctcagcttcttaatataactgccttaaaactttaatcccacttgcccctgttacctaattagagcagatgacccctcccctaatgcctgcggagttgtgcacgtagtagggtcaggccacggcagcctaccggcaatttccggccaacagttaaatgagaacatgaaaacagaaaacggttaaaactgtccctttctgtgtgaagatcacgttccttcccccgcaatgtgcccccagacgcacgtgggtcttcagggggccaggtgcacagacgtccctccacgttcacccctccacccttggactttcttttcgccgtggctgcggcacccttgcgcttttgctggtcactgccatggaggcacacagctgcagagacagagaggacgtgggcggcagagaggactgttgacatccaagcttcctttgtttttttttcctgtccttctctcacctcctaaagtagacttcatttttcctaacaggattagacagtcaaggagtggcttactacatgtgggagcttttggtatgtgacatgcgggctgggcagctgttagagtccaacgtggggcagcacagagagggggccacctccccaggccgtggctgcccacacaccccaattagctgaattcgcgtgtggcagagggaggaaaaggaggcaaacgtgggctgggcaatggcctcacataggaaacagggtcttcctggagatttggtgatggagatgtcaagcaggtggcctctggacgtcaccgttgccctgcatggtggccccagagcagcctctatgaacaacctcgtttccaaaccacagcccacagccggagagtccaggaagacttgcgcactcagagcagaagggtaggagtcctctagacagcctcgcagccgcgccagtcgcccatagacactggctgtgaccgggcgtgctggcagcggcagtgcacagtggccagcactaaccctccctgagaagataaccggctcattcacttcctcccagaagacgcgtggtagcgagtaggcacaggcgtgcacctgctcccgaattactcaccgagacacacgggctgagcagacggccccgtggatggagacaaagagctcttctgaccatatccttcttaacacccgctggcatctcctttcgcgcctccctccctaacctactgacccaccttttgattttagcgcacctgtgattgataggccttccaaagagtcccacgctggcatcaccctccccgaggacggagatgaggagtagtcagcgtgatgccaaaacgcgtcttcttaatccaattctaattctgaatgtttcgtgtgggcttaataccatgtctattaatatatagcctcgatgatgagagagttacaaagaacaaaactccagacacaaacctccaaatttttcagcagaagcactctgcgtcgctgagctgaggtcggctctgcgatccatacgtggccgcacccacacagcacgtgctgtgacgatggctgaacggaaagtgtacactgttcctgaatattgaaataaaacaataaacttttaatggtaaaaaaaaaaaaaaaaaaaaaa

SEQ ID NO: 241 - DNA, 2069 bp, Homo sapiens
catctttgatgagggcagagctcacgttgcattgaagacgaaacctcggggaggtcaggcgctgtctttccttccctccctgctcggcggctccaccacagttgcaacctgcagaggcccggagaacacaaccctcccgagaagcccaggtccagagccaaacccgtcactgaccccccagcccaggcgcccagccactccccaccgctaccatggccgaagacgcagacatgcgcaatgagctggaggagatgcagcgaagggctgaccagttggctgatgagtcgctggaaagcacccgtcgtatgctgcaactggttgaagagagtaaagatgctggtatcaggactttggttatgttggatgaacaaggagaacaactggaacgcattgaggaagggatggaccaaatcaataaggacatgaaagaagcagaaaagaatttgacggacctaggaaaattctgcgggctttgtgtgtgtccctgtaacaagcttaaatcaagtgatgcttacaaaaaagcctggggcaataatcaggacggagtggtggccagccagcctgctcgtgtagtggacgaacgggagcagatggccatcagtggcggcttcatccgcagggtaacaaatgatgcccgagaaaatgaaatggatgaaaacctagagcaggtgagcggcatcatcgggaacctccgtcacatggccctggatatgggcaatgagatcgatacacagaatcgccagatcgacaggatcatggagaaggctgattccaacaaaaccagaattgatgaggccaaccaacgtgcaacaaagatgctgggaagtggttaagtgtgcccacccgtgttctcctccaaatgctgtcgggcaagatagctccttcatgcttttctcatggtattatctagtaggtctgcacacataacacacatcagtccacccccattgtgaatgttgtcctgtgtcatctgtcagcttcccaacaatactttgtgtcttttgttctctcttggtctctttctttccaaaggttgtacatagtggtcatttggtggctctaactccttgaggtcttgagtttcatttttcattttctctcctcggtggcatttgctgaataacaacaatttaggaatgctcaatgtgctgttgattctttcaatccacagtattgttcttgtaaaactgtgacattccacagagttactgccacggtcctttgagtgtcaggctctgaatctctcaaaatgtgccgtctttggttcctcatggctgttatctgtctttatgatttcatgattagacaatgtggaattacataacaggcattgcactaaaagtgatgtgatttatgcatttatgcatgagaactaaatagatttttagattcctacttaaacaaaaactttccatgacagtagcatactgatgagacaacacacacacacacaaaacaacagcaacaacaacagaacaacaacaaagcatgctcagtattgagacactgtcaagattaagttataccagcaaaagtgcagtagtgtcacttttttcctgtcaatatatagagacttctaaatcataatcatccttttttaaaaaaaagaattttaaaaaagatggatttgacacactcaccatttaatcatttccagcaaaatatatgtttggctgaaattatgtcaaatggatgtaatatagggtttgtttgctgcttttgatggctatgttttggagagagcaatcttgctgtgaaacagtgtggatgtaaattttataaggctgactcttactaaccaccatttcccctgtggtttgttatcagtacaattctttgttgcttaatctagagctatgcacaccaaattgctgagatgtttagtagctgataaagaaaccttttaaaaaaataatataaatgaatgaaatataaactgtgagataaatatcattatagcatgtaatattaaattcctcctgtctcctctgtcagtttgtgaagtgattgacattttgtagctagtttaaaattattaaaaattatagactccaaaaaaaaaaaaaaaa

SEQ ID NO: 242 - DNA, 1513 bp, Homo sapiens
gcctcaagaccttgggctgggactggctgagcctggcgggaggcggggtccgagtcaccgcctgccgccgcgcccccggtttctataaattgagcccgcagcctcccgcttcgctctctgctcctcctgttcgacagtcagccgcatcttcttttgcgtcgccaggtgaagacgggcggagagaaacccgggaggctagggacggcctgaaggcggcaggggcgggcgcaggccggatgtgttcgcgccgctgcgggccgagccacatcgctcagacaccatggggaaggtgaaggtcggagtcaacggatttggtcgtattgggcgcctggtcaccagggctgcttttaactctggtaaagtggatattgttgccatcaatgaccccttcattgacctcaactacatggtttacatgttccaatatgattccacccatggcaaattccatggcaccgtcaaggctgagaacgggaagcttgtcatcaatggaaatcccatcaccatcttccaggagcgagatccctccaaaatcaagtggggcgatgctggcgctgagtacgtcgtggagtccactggcgtcttcaccaccatggagaaggctggggctcatttgcaggggggagccaaaagggtcatcatctctgccccctctgctgatgcccccatgttcgtcatgggtgtgaaccatgagaagtatgacaacagcctcaagatcatcagcaatgcctcctgcaccaccaactgcttagcacccctggccaaggtcatccatgacaactttggtatcgtggaaggactcatgaccacagtccatgccatcactgccacccagaagactgtggatggcccctccgggaaactgtggcgtgatggccgcggggctctccagaacatcatccctgcctctactggcgctgccaaggctgtgggcaaggtcatccctgagctgaacgggaagctcactggcatggccttccgtgtccccactgccaacgtgtcagtggtggacctgacctgccgtctagaaaaacctgccaaatatgatgacatcaagaaggtggtgaagcaggcgtcggagggccccctcaagggcatcctgggctacactgagcaccaggtggtctcctctgacttcaacagcgacacccactcctccacctttgacgctggggctggcattgccctcaacgaccactttgtcaagctcatttcctggtatgacaacgaatttggctacagcaacagggtggtggacctcatggcccacatggcctccaaggagtaagacccctggaccaccagccccagcaagagcacaagaggaagagagagaccctcactgctggggagtccctgccacactcagtcccccaccacactgaatctcccctcctcacagttgccatgtagaccccttgaagaggggaggggcctagggagccgcaccttgtcatgtaccatcaataaagtaccctgtgctcaaccagttaaaaaaaaaaaaaaaaaaaaa

SEQ ID NO: 243 - DNA, 299 bp, Homo sapiens
gccgggcgcggtggcgcgtgcctgtagtcccagctactcgggaggctgaggtgggaggatcgcttgagcccaggagttctgggctgtagtgcgctatgccgatcgggtgtccgcactaagttcggcatcaatatggtgacctcccgggagcgggggaccaccaggttgcctaaggaggggtgaaccggcccaggtcggaaacggagcaggtcaaaactcccgtgctgatcagtagtgggatcgcgcctgtgaatagccactgcactccagcctgagcaacatagcgagaccccgtctct